European Patent Application EP 4 592 311 A2, published July 30, 2025. Title: Antibodies. Applicant: Medler Ferro Woodhouse & Mills PLLC. Application EP, filed May 2, 2025. The sequence listing filed with the application follows.

SEQUENCE LISTING (40 sequences)

SEQ ID NO: 1 - protein, 214 aa, Synthetic construct
DIQMTQSPSSLSASVGDRVTITCRASQDVNTAVAWYQQKPGKAPKLLIYSASFLYSGVPSRFSGSRSGTDFTLTISSLQPEDFATYYCQQHYTTPPTFGQGTKVEIKRTVAAPSVFIFPPSDEQLKSGTASVVCLLNNFYPREAKVQWKVDNALQSGNSQESVTEQDSKDSTYSLSSTLTLSKADYEKHKVYACEVTHQGLSSPVTKSFNRGEC

SEQ ID NO: 2 - protein, 450 aa, Synthetic construct
EVQLVESGGGLVQPGGSLRLSCAASGFNIKDTYIHWVRQAPGKGLEWVARIYPTNGYTRYADSVKGRFTISADTSKNTAYLQMNSLRAEDTAVYYCSRWGGDGFYAMDYWGQGTLVTVSSASTKGPSVFPLAPSSKSTSGGTAALGCLVKDYFPEPVTVSWNSGALTSGVHTFPAVLQSSGLYSLSSVVTVPSSSLGTQTYICNVNHKPSNTKVDKKVEPKSCDKTHTCPPCPAPELLGGPSVFLFPPKPKDTLMISRTPEVTCVVVDVSHEDPEVKFNWYVDGVEVHNAKTKPREEQYNSTYRVVSVLTVLHQDWLNGKEYKCKVSNKALPAPIEKTISKAKGQPREPQVYTLPPSRDELTKNQVSLTCLVKGFYPSDIAVEWESNGQPENNYKTTPPVLDSDGSFFLYSKLTVDKSRWQQGNVFSCSVMHEALHNHYTQKSLSLSPGK

SEQ ID NO: 3 - protein, 450 aa, Synthetic construct
EVQLVESGGGLVQPGGSLRLSCAASGFNIKDTYIHWVRQAPGKGLEWVARIYPTNGYTRYADSVKGRFTISADTSKNTAYLQMNSLRAEDTAVYYCSRWGGDGFYAMDYWGQGTLVTVSSASTKGPSVFPLAPSSKSTCGGTAALGCLVKDYFPEPVTVSWNSGALTSGVHTFPAVLQSSGLYSLSSVVTVPSSSLGTQTYICNVNHKPSNTKVDKRVEPKSCDKTHTCPPCPAPELLGGPSVFLFPPKPKDTLMISRTPEVTCVVVDVSHEDPEVKFNWYVDGVEVHNAKTKPREEQYNSTYRVVSVLTVLHQDWLNGKEYKCKVSNKALPAPIEKTISKAKGQPREPQVYTLPPSREEMTKNQVSLTCLVKGFYPSDIAVEWESNGQPENNYKTTPPVLDSDGSFFLYSKLTVDKSRWQQGNVFSCSVMHEALHNHYTQKSLSLSPGK

SEQ ID NO: 4 - protein, 450 aa, Synthetic construct
EVQLVESGGGLVQPGGSLRLSCAASGFNIKDTYIHWVRQAPGKGLEWVARIYPTNGYTRYADSVKGRFTISADTSKNTAYLQMNSLRAEDTAVYYCSRWGGDGFYAMDYWGQGTLVTVSSASTKGPSVFPLAPSSKSTSGGTAALGCLVKDYFPEPVTVCWNSGALTSGVHTFPAVLQSSGLYSLSSVVTVPSSSLGTQTYICNVNHKPSNTKVDKRVEPKSCDKTHTCPPCPAPELLGGPSVFLFPPKPKDTLMISRTPEVTCVVVDVSHEDPEVKFNWYVDGVEVHNAKTKPREEQYNSTYRVVSVLTVLHQDWLNGKEYKCKVSNKALPAPIEKTISKAKGQPREPQVYTLPPSREEMTKNQVSLTCLVKGFYPSDIAVEWESNGQPENNYKTTPPVLDSDGSFFLYSKLTVDKSRWQQGNVFSCSVMHEALHNHYTQKSLSLSPGK

SEQ ID NO: 5 - protein, 450 aa, Synthetic construct
EVQLVESGGGLVQPGGSLRLSCAASGFNIKDTYIHWVRQAPGKGLEWVARIYPTNGYTRYADSVKGRFTISADTSKNTAYLQMNSLRAEDTAVYYCSRWGGDGFYAMDYWGQGTLVTVSSASTKGPSVFPLAPSSKSTSGGTAALGCLVKDYFPEPVTVSWNSGALTCGVHTFPAVLQSSGLYSLSSVVTVPSSSLGTQTYICNVNHKPSNTKVDKRVEPKSCDKTHTCPPCPAPELLGGPSVFLFPPKPKDTLMISRTPEVTCVVVDVSHEDPEVKFNWYVDGVEVHNAKTKPREEQYNSTYRVVSVLTVLHQDWLNGKEYKCKVSNKALPAPIEKTISKAKGQPREPQVYTLPPSREEMTKNQVSLTCLVKGFYPSDIAVEWESNGQPENNYKTTPPVLDSDGSFFLYSKLTVDKSRWQQGNVFSCSVMHEALHNHYTQKSLSLSPGK

SEQ ID NO: 6 - protein, 450 aa, synthetic construct
EVQLVESGGGLVQPGGSLRLSCAASGFNIKDTYIHWVRQAPGKGLEWVARIYPTNGYTRYADSVKGRFTISADTSKNTAYLQMNSLRAEDTAVYYCSRWGGDGFYAMDYWGQGTLVTVSSASTKGPSVFPLAPSSKSTSGGTAALGCLVKDYFPEPVTVSWNSGALTSGCHTFPAVLQSSGLYSLSSVVTVPSSSLGTQTYICNVNHKPSNTKVDKRVEPKSCDKTHTCPPCPAPELLGGPSVFLFPPKPKDTLMISRTPEVTCVVVDVSHEDPEVKFNWYVDGVEVHNAKTKPREEQYNSTYRVVSVLTVLHQDWLNGKEYKCKVSNKALPAPIEKTISKAKGQPREPQVYTLPPSREEMTKNQVSLTCLVKGFYPSDIAVEWESNGQPENNYKTTPPVLDSDGSFFLYSKLTVDKSRWQQGNVFSCSVMHEALHNHYTQKSLSLSPGK

SEQ ID NO: 7 - protein, 450 aa, synthetic construct
EVQLVESGGGLVQPGGSLRLSCAASGFNIKDTYIHWVRQAPGKGLEWVARIYPTNGYTRYADSVKGRFTISADTSKNTAYLQMNSLRAEDTAVYYCSRWGGDGFYAMDYWGQGTLVTVSSASTKGPSVFPLAPSSKSTSGGTAALGCLVKDYFPEPVTVSWNSGALTSGVHTFPACLQSSGLYSLSSVVTVPSSSLGTQTYICNVNHKPSNTKVDKRVEPKSCDKTHTCPPCPAPELLGGPSVFLFPPKPKDTLMISRTPEVTCVVVDVSHEDPEVKFNWYVDGVEVHNAKTKPREEQYNSTYRVVSVLTVLHQDWLNGKEYKCKVSNKALPAPIEKTISKAKGQPREPQVYTLPPSREEMTKNQVSLTCLVKGFYPSDIAVEWESNGQPENNYKTTPPVLDSDGSFFLYSKLTVDKSRWQQGNVFSCSVMHEALHNHYTQKSLSLSPGK

SEQ ID NO: 8 - protein, 450 aa, Synthetic construct
EVQLVESGGGLVQPGGSLRLSCAASGFNIKDTYIHWVRQAPGKGLEWVARIYPTNGYTRYADSVKGRFTISADTSKNTAYLQMNSLRAEDTAVYYCSRWGGDGFYAMDYWGQGTLVTVSSASTKGPSVFPLAPSSKSTSGGTAALGCLVKDYFPEPVTVSWNSGALTSGVHTFPAVLQSSGLYSLSSVVCVPSSSLGTQTYICNVNHKPSNTKVDKRVEPKSCDKTHTCPPCPAPELLGGPSVFLFPPKPKDTLMISRTPEVTCVVVDVSHEDPEVKFNWYVDGVEVHNAKTKPREEQYNSTYRVVSVLTVLHQDWLNGKEYKCKVSNKALPAPIEKTISKAKGQPREPQVYTLPPSREEMTKNQVSLTCLVKGFYPSDIAVEWESNGQPENNYKTTPPVLDSDGSFFLYSKLTVDKSRWQQGNVFSCSVMHEALHNHYTQKSLSLSPGK

SEQ ID NO: 9 - protein, 450 aa, Synthetic construct
EVQLVESGGGLVQPGGSLRLSCAASGFNIKDTYIHWVRQAPGKGLEWVARIYPTNGYTRYADSVKGRFTISADTSKNTAYLQMNSLRAEDTAVYYCSRWGGDGFYAMDYWGQGTLVTVSSASTKGPSVFPLAPSSKSTSGGTAALGCLVKDYFPEPVTVSWNSGALTSGVHTFPAVLQSSGLYSLSSVVTVPSSSLGTQCYICNVNHKPSNTKVDKRVEPKSCDKTHTCPPCPAPELLGGPSVFLFPPKPKDTLMISRTPEVTCVVVDVSHEDPEVKFNWYVDGVEVHNAKTKPREEQYNSTYRVVSVLTVLHQDWLNGKEYKCKVSNKALPAPIEKTISKAKGQPREPQVYTLPPSREEMTKNQVSLTCLVKGFYPSDIAVEWESNGQPENNYKTTPPVLDSDGSFFLYSKLTVDKSRWQQGNVFSCSVMHEALHNHYTQKSLSLSPGK

SEQ ID NO: 10 - protein, 450 aa, Synthetic construct
EVQLVESGGGLVQPGGSLRLSCAASGFNIKDTYIHWVRQAPGKGLEWVARIYPTNGYTRYADSVKGRFTISADTSKNTAYLQMNSLRAEDTAVYYCSRWGGDGFYAMDYWGQGTLVTVSSASTKGPSVFPLAPSSKSTSGGTAALGCLVKDYFPEPVTVSWNSGALTSGVHTFPAVLQSSGLYSLSSVVTVPSSSLGTQTYICNVNHKPSNTKVDKRVEPKSCDKTHTCPPCPAPELLGGPSVFLFPPKPKDTLMISRTPEVTCVVVDVSHEDPEVKFNWYVDGVEVHNAKTKPREEQYNSTYRVVSVLTVLHQDWLNGKEYKCKVSNKALPAPIEKTISKAKGQPREPQVYTLPPSREEMTKNQVSLTCLVKGFYPSDIAVEWESNGQPENNYKTTPPVLDSDGSFFLYSKLTVDKSRWQQGNVFSCSVMHEALHNHYTQKCLSLSPGK

SEQ ID NO: 11 - protein, 450 aa, synthetic construct
EVQLVESGGGLVQPGGSLRLSCAASGFNIKDTYIHWVRQAPGKGLEWVARIYPTNGYTRYADSVKGRFTISADTSKNTAYLQMNSLRAEDTAVYYCSRWGGDGFYAMDYWGQGTLVTVSSASTKGPSVFPLAPSSKSTSGGTAALGCLVKDYFPEPVTVSWNSGALTSGVHTFPAVLQSSGLYSLSSVVTVPSSSLGTQTYICNVNHKPSNTKVDKRVEPKSCDKTHTCPPCPAPELLGGPSVFLFPPKPKDTLMISRTPEVTCVVVDVSHEDPEVKFNWYVDGVEVHNAKTKPREEQYNSTYRVVSVLTVLHQDWLNGKEYKCKVSNKALPAPIEKTISKAKGQPREPQVYTLPPSREEMTKNQVSLTCLVKGFYPSDIAVEWESNGQPENNYKTTPPVLDSDGSFFLYSKLTVDKSRWQQGNVFSCSVMHEALHNHYTQKSLCLSPGK

SEQ ID NO: 12 - protein, 450 aa, synthetic construct
EVQLVESGGGLVQPGGSLRLSCAASGFNIKDTYIHWVRQAPGKGLEWVARIYPTNGYTRYADSVKGRFTISADTSKNTAYLQMNSLRAEDTAVYYCSRWGGDGFYAMDYWGQGTLVTVSSASTKGPSVFPLAPSSKSTSGGTAALGCLVKDYFPEPVTVSWNSGALTSGVHTFPAVLQSSGLYSLSSVVTVPSSSLGTQTYICNVNHKPSNTKVDKRVEPKSCDKTHTCPPCPAPELLGGPSVFLFPPKPKDTLMISRTPEVTCVVVDVSHEDPEVKFNWYVDGVEVHNAKTKPREEQYNSTYRVVSVLTVLHQDWLNGKEYKCKVSNKALPAPIEKTISKAKGQPREPQVYTLPPSREEMTKNQVSLTCLVKGFYPSDIAVEWESNGQPENNYKTTPPVLDSDGSFFLYSKLTVDKSRWQQGNVFSCSVMHEALHNHYTQKSLSLCPGK

SEQ ID NO: 13 - protein, 214 aa, Synthetic construct
DIQMTQSPSSLSASVGDRVTITCRASQDVNTAVAWYQQKPGKAPKLLIYSASFLYSGVPSRFSGSRSGTDFTLTISSLQPEDFATYYCQQHYTTPPTFGQGTKVEIKRTVAAPSVFIFPPSDEQLKSGTASVVCLLNNFYPREAKVQWKVDNALQSGNSQESVTEQDSKDCTYSLSSTLTLSKADYEKHKVYACEVTHQGLSSPVTKSFNRGEC

SEQ ID NO: 14 - protein, 214 aa, Synthetic construct
DIQMTQSPSSLSASVGDRVTITCRASQDVNTAVAWYQQKPGKAPKLLIYSASFLYSGVPSRFSGSRSGTDFTLTISSLQPEDFATYYCQQHYTTPPTFGQGTKVEIKRTVAAPSVFIFPPSDEQLKSGTASVVCLLNNFYPREAKVQWKVDNALQSGNSQESVTEQDSKDSTYSLSSTLCLSKADYEKHKVYACEVTHQGLSSPVTKSFNRGEC

SEQ ID NO: 15 - protein, 214 aa, synthetic construct
DIQMTQSPSSLSASVGDRVTITCRASQDVNTAVAWYQQKPGKAPKLLIYSASFLYSGVPSRFSGSRSGTDFTLTISSLQPEDFATYYCQQHYTTPPTFGQGTKVEIKRTVAAPSVFIFPPSDEQLKSGTASVVCLLNNFYPREAKVQWKVDNALQSGNSQESVTEQDSKDSTYSLSSTLTLCKADYEKHKVYACEVTHQGLSSPVTKSFNRGEC

SEQ ID NO: 16 - protein, 214 aa, Synthetic construct
DIQMTQSPSSLSASVGDRVTITCRASQDVNTAVAWYQQKPGKAPKLLIYSASFLYSGVPSRFSGSRSGTDFTLTISSLQPEDFATYYCQQHYTTPPTFGQGTKVEIKRTVAAPSVFIFPPSDEQLKSGTASVVCLLNNFYPREAKVQWKVDNALQSGNSQESVTEQDSKDSTYSLSSTLTLSKCDYEKHKVYACEVTHQGLSSPVTKSFNRGEC

SEQ ID NO: 17 - protein, 214 aa, Synthetic construct
DIQMTQSPSSLSASVGDRVTITCRASQDVNTAVAWYQQKPGKAPKLLIYSASFLYSGVPSRFSGSRSGTDFTLTISSLQPEDFATYYCQQHYTTPPTFGQGTKVEIKRTVAAPSVFIFPPSDEQLKSGTASVVCLLNNFYPREAKVQWKVDNALQSGNSQESVTEQDSKDSTYSLSSTLTLSKADYEKHKCYACEVTHQGLSSPVTKSFNRGEC

SEQ ID NO: 18 - protein, 214 aa, Synthetic construct
DIQMTQSPSSLSASVGDRVTITCRASQDVNTAVAWYQQKPGKAPKLLIYSASFLYSGVPSRFSGSRSGTDFTLTISSLQPEDFATYYCQQHYTTPPTFGQGTKVEIKRTVAAPSVFIFPPSDEQLKSGTASVVCLLNNFYPREAKVQWKVDNALQSGNSQESVTEQDSKDSTYSLSSTLTLSKADYEKHKVYACEVTHQGLCSPVTKSFNRGEC

SEQ ID NO: 19 - protein, 214 aa, Synthetic construct
DIQMTQSPSSLSASVGDRVTITCRASQDVNTAVAWYQQKPGKAPKLLIYSASFLYSGVPSRFSGSRSGTDFTLTISSLQPEDFATYYCQQHYTTPPTFGQGTKVEIKRTVAAPSVFIFPPSDEQLKSGTASVVCLLNNFYPREAKVQWKVDNALQSGNSQESVTEQDSKDSTYSLSSTLTLSKADYEKHKVYACEVTHQGLSCPVTKSFNRGEC

SEQ ID NO: 20 - protein, 214 aa, Synthetic construct
DIQMTQSPSSLSASVGDRVTITCRASQDVNTAVAWYQQKPGKAPKLLIYSASFLYSGVPSRFSGSRSGTDFTLTISSLQPEDFATYYCQQHYTTPPTFGQGTKVEIKRTVAAPSVFIFPPSDEQLKSGTASVVCLLNNFYPREAKVQWKVDNALQSGNSQESVTEQDSKDSTYSLSSTLTLSKADYEKHKVYACEVTHQGLSSPVCKSFNRGEC

SEQ ID NO: 21 - protein, 214 aa, Synthetic construct
DIQMTQSPSSLSASVGDRVTITCRASQDVNTAVAWYQQKPGKAPKLLIYSASFLYSGVPSRFSGSRSGTDFTLTISSLQPEDFATYYCQQHYTTPPTFGQGTKVEIKRTVAAPSVFIFPPSDEQLKSGTASVVCLLNNFYPREAKVQWKVDNALQSGNSQESVTEQDSKDSTYSLSSTLTLSKADYEKHKVYACEVTHQGLSSPVTKCFNRGEC

SEQ ID NO: 22 - protein, 21 aa, Synthetic construct
FPLAPSSKSTXGGTAALGCLV

SEQ ID NO: 23 - protein, 21 aa, Synthetic construct
KDYFPEPVTVXWNSGALTSGV

SEQ ID NO: 24 - protein, 21 aa, Synthetic construct
TVSWNSGALTXGVHTFPAVLQ

SEQ ID NO: 25 - protein, 21 aa, synthetic construct
SWNSGALTSGXHTFPAVLQSS

SEQ ID NO: 26 - protein, 21 aa, Synthetic construct
LTSGVHTFPAXLQSSGLYSLS

SEQ ID NO: 27 - protein, 21 aa, Synthetic construct
SGLYSLSSVVXVPSSSLGTQT

SEQ ID NO: 28 - protein, 21 aa, Synthetic construct
TVPSSSLGTQXYICNVNHKPS

SEQ ID NO: 29 - protein, 18 aa, Synthetic construct
EALHNHYTQKXLSLSPGK

SEQ ID NO: 30 - protein, 18 aa, Synthetic construct
EALHNHYTQKSLXLSPGK

SEQ ID NO: 31 - protein, 18 aa, Synthetic construct
EALHNHYTQKSLSLXPGK

SEQ ID NO: 32 - protein, 21 aa, Synthetic construct
ESVTEQDSKDXTYSLSSTLTL

SEQ ID NO: 33 - protein, 21 aa, Synthetic construct
DSTYSLSSTLXLSKADYEKHK

SEQ ID NO: 34 - protein, 21 aa, Synthetic construct
TYSLSSTLTLXKADYEKHKVY

SEQ ID NO: 35 - protein, 21 aa, synthetic construct
SLSSTLTLSKXDYEKHKVYAC

SEQ ID NO: 36 - protein, 21 aa, synthetic construct
LSKADYEKHKXYACEVTHQGL

SEQ ID NO: 37 - protein, 21 aa, Synthetic construct
YACEVTHQGLXSPVTKSFNRG

SEQ ID NO: 38 - protein, 21 aa, Synthetic construct
ACEVTHQGLSXPVTKSFNRGE

SEQ ID NO: 39 - protein, 19 aa, Synthetic construct
VTHQGLSSPVXKSFNRGEC

SEQ ID NO: 40 - protein, 19 aa, synthetic construct
VTHQGLSSPVTKXFNRGEC